European Patent Specification EP 3 749 770 B1, published October 15, 2025. Title: TETHERED INTERLEUKIN-15 AND INTERLEUKIN-21. Applicant: THE UNITED STATES OF AMERICA, AS REPRESENTED BY THE SECRETARY, DEPARTMENT OF HEALTH AND HUMAN SERVICES Hinrichs, Christian  S. Jin, Benjamin  Y. The sequence listing filed with the application follows.

SEQUENCE LISTING (44 sequences)

SEQ ID NO: 1 - protein, 18 aa, Homo sapiens
MDWTWILFLVAAATRVHS

SEQ ID NO: 2 - protein, 133 aa, Homo sapiens [sequence omitted]

SEQ ID NO: 3 - protein, 114 aa, Homo sapiens
NWVNVISDLKKIEDLIQSMHIDATLYTESDVHPSCKVTAMKCFLLELQVISLESGDASIHDTVENLIILANNSLSSNGNVTESGCKECEELEEKNIKEFLQSFVHIVQMFINTS

SEQ ID NO: 4 - protein, 21 aa, Homo sapiens
IYIWAPLAGTCGVLLLSLVIT

SEQ ID NO: 5 - protein, 46 aa, Homo sapiens
LLPSWAITLISVNGIFVICCLTYCFAPRCRERRRNERLRRESVRPV

SEQ ID NO: 6 - protein, 9 aa, porcine teschovirus-1 2A
  MISC_FEATURE (5)..(5): X is any naturally occurring amino acid residue.
GDVEXNPGP

SEQ ID NO: 7 - protein, 22 aa, porcine teschovirus-1 2A
GSGATNFSLLKQAGDVEENPGP

SEQ ID NO: 8 - protein, 23 aa, equine rhinitis A virus 2a
GSGQCTNYALLKLAGDVESNPGP

SEQ ID NO: 9 - protein, 21 aa, thosea asigna virus 2A
GSGEGRGSLLTCGDVEENPGP

SEQ ID NO: 10 - protein, 4 aa, Artificial Sequence
  synthetic
  MISC_FEATURE (2)..(2): X is any naturally occurring amino acid.
  MISC_FEATURE (3)..(3): X is arginine or lysine.
RXXR

SEQ ID NO: 11 - protein, 27 aa, Artificial Sequence
  synthetic
RAKRSGSGATNFSLLKQAGDVEENPGP

SEQ ID NO: 12 - protein, 27 aa, Artificial Sequence
  synthetic
SGGGGSGGGGSGGGGSGGGGSGGGSLQ

SEQ ID NO: 13 - protein, 18 aa, Artificial Sequence
  synthetic
GSTSGSGKPGSGEGSTKG

SEQ ID NO: 14 - protein, 45 aa, Artificial Sequence
  synthetic
GGGGSGGGGSGGGGSGGGGSGGGGSGGGGSGGGGSGGGGSGGGGS

SEQ ID NO: 15 - protein, 46 aa, Artificial Sequence
  synthetic
AEAAAKEAAAKEAAAKEAAAKALEAEAAAKEAAAKEAAAKEAAAKA

SEQ ID NO: 16 - protein, 48 aa, Artificial Sequence
  synthetic
SGGGGSGGGGSGGGGSGGGGSGGGGSGGGGSGGGGSGGGGSGGGGSLQ

SEQ ID NO: 17 - protein, 61 aa, Artificial Sequence
  synthetic
AGGGSGGGGSGGGGSGGGGSGGGGSGGGGSGGGGSGGGGSGGGGSGGGSGGGGSGGGGSAS

SEQ ID NO: 18 - protein, 237 aa, Artificial Sequence
  synthetic
ITCPPPMSVEHADIWVKSYSLYSRERYICNSGFKRKAGTSSLTECVLNKATNVAHWTTPSLKCIRDPALVHQRPAPPSTVTTAGVTPQPESLSPSGKEPAASSPSSNNTAATTAAIVPGSQLMPSKSPSTGTTEISSHESSHGTPSQTTAKNWELTASASHQPPGVYPQGHSDTTVAISTSTVLLCGLSAVSLLACYLKSRQTPPLASVEMEAMEALPVTWGTSSRDEDLENCSHHL

SEQ ID NO: 19 - protein, 180 aa, Artificial Sequence
  synthetic
MDWTWILFLVAAATRVHSNWVNVISDLKKIEDLIQSMHIDATLYTESDVHPSCKVTAMKCFLLELQVISLESGDASIHDTVENLIILANNSLSSNGNVTESGCKECEELEEKNIKEFLQSFVHIVQMFINTSSGGGGSGGGGSGGGGSGGGGSGGGSLQIYIWAPLAGTCGVLLLSLVIT

SEQ ID NO: 20 - protein, 171 aa, Artificial Sequence
  synthetic
MDWTWILFLVAAATRVHSNWVNVISDLKKIEDLIQSMHIDATLYTESDVHPSCKVTAMKCFLLELQVISLESGDASIHDTVENLIILANNSLSSNGNVTESGCKECEELEEKNIKEFLQSFVHIVQMFINTSGSTSGSGKPGSGEGSTKGIYIWAPLAGTCGVLLLSLVIT

SEQ ID NO: 21 - protein, 396 aa, Artificial Sequence
  synthetic
MDWTWILFLVAAATRVHSNWVNVISDLKKIEDLIQSMHIDATLYTESDVHPSCKVTAMKCFLLELQVISLESGDASIHDTVENLIILANNSLSSNGNVTESGCKECEELEEKNIKEFLQSFVHIVQMFINTSSGGGGSGGGGSGGGGSGGGGSGGGSLQITCPPPMSVEHADIWVKSYSLYSRERYICNSGFKRKAGTSSLTECVLNKATNVAHWTTPSLKCIRDPALVHQRPAPPSTVTTAGVTPQPESLSPSGKEPAASSPSSNNTAATTAAIVPGSQLMPSKSPSTGTTEISSHESSHGTPSQTTAKNWELTASASHQPPGVYPQGHSDTTVAISTSTVLLCGLSAVSLLACYLKSRQTPPLASVEMEAMEALPVTWGTSSRDEDLENCSHHL

SEQ ID NO: 22 - protein, 198 aa, Artificial Sequence
  synthetic
MDWTWILFLVAAATRVHSNWVNVISDLKKIEDLIQSMHIDATLYTESDVHPSCKVTAMKCFLLELQVISLESGDASIHDTVENLIILANNSLSSNGNVTESGCKECEELEEKNIKEFLQSFVHIVQMFINTSGGGGSGGGGSGGGGSGGGGSGGGGSGGGGSGGGGSGGGGSGGGGSIYIWAPLAGTCGVLLLSLVIT

SEQ ID NO: 23 - protein, 132 aa, Artificial Sequence
  synthetic
MDWTWILFLVAAATRVHSNWVNVISDLKKIEDLIQSMHIDATLYTESDVHPSCKVTAMKCFLLELQVISLESGDASIHDTVENLIILANNSLSSNGNVTESGCKECEELEEKNIKEFLQSFVHIVQMFINTS

SEQ ID NO: 24 - protein, 199 aa, Artificial Sequence
  synthetic
MDWTWILFLVAAATRVHSQGQDRHMIRMRQLIDIVDQLKNYVNDLVPEFLPAPEDVETNCEWSAFSCFQKAQLKSANTGNNERIINVSIKKLKRKPPSTNAGRRQKHRLTCPSCDSYEKKPPKEFLERFKSLLQKMIHQHLSSRTHGSEDSSGGGGSGGGGSGGGGSGGGGSGGGSLQIYIWAPLAGTCGVLLLSLVIT

SEQ ID NO: 25 - protein, 190 aa, Artificial Sequence
  synthetic
MDWTWILFLVAAATRVHSQGQDRHMIRMRQLIDIVDQLKNYVNDLVPEFLPAPEDVETNCEWSAFSCFQKAQLKSANTGNNERIINVSIKKLKRKPPSTNAGRRQKHRLTCPSCDSYEKKPPKEFLERFKSLLQKMIHQHLSSRTHGSEDSGSTSGSGKPGSGEGSTKGIYIWAPLAGTCGVLLLSLVIT

SEQ ID NO: 26 - protein, 217 aa, Artificial Sequence
  synthetic
MDWTWILFLVAAATRVHSQGQDRHMIRMRQLIDIVDQLKNYVNDLVPEFLPAPEDVETNCEWSAFSCFQKAQLKSANTGNNERIINVSIKKLKRKPPSTNAGRRQKHRLTCPSCDSYEKKPPKEFLERFKSLLQKMIHQHLSSRTHGSEDSGGGGSGGGGSGGGGSGGGGSGGGGSGGGGSGGGGSGGGGSGGGGSIYIWAPLAGTCGVLLLSLVIT

SEQ ID NO: 27 - protein, 218 aa, Artificial Sequence
  synthetic
MDWTWILFLVAAATRVHSQGQDRHMIRMRQLIDIVDQLKNYVNDLVPEFLPAPEDVETNCEWSAFSCFQKAQLKSANTGNNERIINVSIKKLKRKPPSTNAGRRQKHRLTCPSCDSYEKKPPKEFLERFKSLLQKMIHQHLSSRTHGSEDSAEAAAKEAAAKEAAAKEAAAKALEAEAAAKEAAAKEAAAKEAAAKAIYIWAPLAGTCGVLLLSLVIT

SEQ ID NO: 28 - protein, 220 aa, Artificial Sequence
  synthetic
MDWTWILFLVAAATRVHSQGQDRHMIRMRQLIDIVDQLKNYVNDLVPEFLPAPEDVETNCEWSAFSCFQKAQLKSANTGNNERIINVSIKKLKRKPPSTNAGRRQKHRLTCPSCDSYEKKPPKEFLERFKSLLQKMIHQHLSSRTHGSEDSSGGGGSGGGGSGGGGSGGGGSGGGGSGGGGSGGGGSGGGGSGGGGSLQIYIWAPLAGTCGVLLLSLVIT

SEQ ID NO: 29 - protein, 233 aa, Artificial Sequence
  synthetic
MDWTWILFLVAAATRVHSQGQDRHMIRMRQLIDIVDQLKNYVNDLVPEFLPAPEDVETNCEWSAFSCFQKAQLKSANTGNNERIINVSIKKLKRKPPSTNAGRRQKHRLTCPSCDSYEKKPPKEFLERFKSLLQKMIHQHLSSRTHGSEDSAGGGSGGGGSGGGGSGGGGSGGGGSGGGGSGGGGSGGGGSGGGGSGGGSGGGGSGGGGSASIYIWAPLAGTCGVLLLSLVIT

SEQ ID NO: 30 - protein, 245 aa, Artificial Sequence
  synthetic
MDWTWILFLVAAATRVHSQGQDRHMIRMRQLIDIVDQLKNYVNDLVPEFLPAPEDVETNCEWSAFSCFQKAQLKSANTGNNERIINVSIKKLKRKPPSTNAGRRQKHRLTCPSCDSYEKKPPKEFLERFKSLLQKMIHQHLSSRTHGSEDSSGGGGSGGGGSGGGGSGGGGSGGGGSGGGGSGGGGSGGGGSGGGGSLQLLPSWAITLISVNGIFVICCLTYCFAPRCRERRRNERLRRESVRPV

SEQ ID NO: 31 - protein, 205 aa, Artificial Sequence
  synthetic
MDWTWILFLVAAATRVHSNWVNVISDLKKIEDLIQSMHIDATLYTESDVHPSCKVTAMKCFLLELQVISLESGDASIHDTVENLIILANNSLSSNGNVTESGCKECEELEEKNIKEFLQSFVHIVQMFINTSSGGGGSGGGGSGGGGSGGGGSGGGSLQLLPSWAITLISVNGIFVICCLTYCFAPRCRERRRNERLRRESVRPV

SEQ ID NO: 32 - protein, 447 aa, Artificial Sequence
  synthetic
MDWTWILFLVAAATRVHSQGQDRHMIRMRQLIDIVDQLKNYVNDLVPEFLPAPEDVETNCEWSAFSCFQKAQLKSANTGNNERIINVSIKKLKRKPPSTNAGRRQKHRLTCPSCDSYEKKPPKEFLERFKSLLQKMIHQHLSSRTHGSEDSSGGGGSGGGGSGGGGSGGGGSGGGGSGGGGSGGGGSGGGGSGGGGSLQIYIWAPLAGTCGVLLLSLVITGSGATNFSLLKQAGDVEENPGPMDWTWILFLVAAATRVHSNWVNVISDLKKIEDLIQSMHIDATLYTESDVHPSCKVTAMKCFLLELQVISLESGDASIHDTVENLIILANNSLSSNGNVTESGCKECEELEEKNIKEFLQSFVHIVQMFINTSSGGGGSGGGGSGGGGSGGGGSGGGSLQLLPSWAITLISVNGIFVICCLTYCFAPRCRERRRNERLRRESVRPV

SEQ ID NO: 33 - protein, 448 aa, Artificial Sequence
  synthetic
MDWTWILFLVAAATRVHSQGQDRHMIRMRQLIDIVDQLKNYVNDLVPEFLPAPEDVETNCEWSAFSCFQKAQLKSANTGNNERIINVSIKKLKRKPPSTNAGRRQKHRLTCPSCDSYEKKPPKEFLERFKSLLQKMIHQHLSSRTHGSEDSSGGGGSGGGGSGGGGSGGGGSGGGGSGGGGSGGGGSGGGGSGGGGSLQIYIWAPLAGTCGVLLLSLVITGSGQCTNYALLKLAGDVESNPGPMDWTWILFLVAAATRVHSNWVNVISDLKKIEDLIQSMHIDATLYTESDVHPSCKVTAMKCFLLELQVISLESGDASIHDTVENLIILANNSLSSNGNVTESGCKECEELEEKNIKEFLQSFVHIVQMFINTSSGGGGSGGGGSGGGGSGGGGSGGGSLQLLPSWAITLISVNGIFVICCLTYCFAPRCRERRRNERLRRESVRPV

SEQ ID NO: 34 - protein, 446 aa, Artificial Sequence
  synthetic
MDWTWILFLVAAATRVHSQGQDRHMIRMRQLIDIVDQLKNYVNDLVPEFLPAPEDVETNCEWSAFSCFQKAQLKSANTGNNERIINVSIKKLKRKPPSTNAGRRQKHRLTCPSCDSYEKKPPKEFLERFKSLLQKMIHQHLSSRTHGSEDSSGGGGSGGGGSGGGGSGGGGSGGGGSGGGGSGGGGSGGGGSGGGGSLQIYIWAPLAGTCGVLLLSLVITGSGEGRGSLLTCGDVEENPGPMDWTWILFLVAAATRVHSNWVNVISDLKKIEDLIQSMHIDATLYTESDVHPSCKVTAMKCFLLELQVISLESGDASIHDTVENLIILANNSLSSNGNVTESGCKECEELEEKNIKEFLQSFVHIVQMFINTSSGGGGSGGGGSGGGGSGGGGSGGGSLQLLPSWAITLISVNGIFVICCLTYCFAPRCRERRRNERLRRESVRPV

SEQ ID NO: 35 - protein, 452 aa, Artificial Sequence
  synthetic
MDWTWILFLVAAATRVHSQGQDRHMIRMRQLIDIVDQLKNYVNDLVPEFLPAPEDVETNCEWSAFSCFQKAQLKSANTGNNERIINVSIKKLKRKPPSTNAGRRQKHRLTCPSCDSYEKKPPKEFLERFKSLLQKMIHQHLSSRTHGSEDSSGGGGSGGGGSGGGGSGGGGSGGGGSGGGGSGGGGSGGGGSGGGGSLQIYIWAPLAGTCGVLLLSLVITRAKRSGSGATNFSLLKQAGDVEENPGPMDWTWILFLVAAATRVHSNWVNVISDLKKIEDLIQSMHIDATLYTESDVHPSCKVTAMKCFLLELQVISLESGDASIHDTVENLIILANNSLSSNGNVTESGCKECEELEEKNIKEFLQSFVHIVQMFINTSSGGGGSGGGGSGGGGSGGGGSGGGSLQLLPSWAITLISVNGIFVICCLTYCFAPRCRERRRNERLRRESVRPV

SEQ ID NO: 36 - protein, 473 aa, Artificial Sequence
  synthetic
MDWTWILFLVAAATRVHSQGQDRHMIRMRQLIDIVDQLKNYVNDLVPEFLPAPEDVETNCEWSAFSCFQKAQLKSANTGNNERIINVSIKKLKRKPPSTNAGRRQKHRLTCPSCDSYEKKPPKEFLERFKSLLQKMIHQHLSSRTHGSEDSSGGGGSGGGGSGGGGSGGGGSGGGGSGGGGSGGGGSGGGGSGGGGSLQLLPSWAITLISVNGIFVICCLTYCFAPRCRERRRNERLRRESVRPVGSGQCTNYALLKLAGDVESNPGPMDWTWILFLVAAATRVHSNWVNVISDLKKIEDLIQSMHIDATLYTESDVHPSCKVTAMKCFLLELQVISLESGDASIHDTVENLIILANNSLSSNGNVTESGCKECEELEEKNIKEFLQSFVHIVQMFINTSSGGGGSGGGGSGGGGSGGGGSGGGSLQLLPSWAITLISVNGIFVICCLTYCFAPRCRERRRNERLRRESVRPV

SEQ ID NO: 37 - protein, 477 aa, Artificial Sequence
  synthetic
MDWTWILFLVAAATRVHSQGQDRHMIRMRQLIDIVDQLKNYVNDLVPEFLPAPEDVETNCEWSAFSCFQKAQLKSANTGNNERIINVSIKKLKRKPPSTNAGRRQKHRLTCPSCDSYEKKPPKEFLERFKSLLQKMIHQHLSSRTHGSEDSSGGGGSGGGGSGGGGSGGGGSGGGGSGGGGSGGGGSGGGGSGGGGSLQLLPSWAITLISVNGIFVICCLTYCFAPRCRERRRNERLRRESVRPVRAKRSGSGATNFSLLKQAGDVEENPGPMDWTWILFLVAAATRVHSNWVNVISDLKKIEDLIQSMHIDATLYTESDVHPSCKVTAMKCFLLELQVISLESGDASIHDTVENLIILANNSLSSNGNVTESGCKECEELEEKNIKEFLQSFVHIVQMFINTSSGGGGSGGGGSGGGGSGGGGSGGGSLQLLPSWAITLISVNGIFVICCLTYCFAPRCRERRRNERLRRESVRPV

SEQ ID NO: 38 - protein, 27 aa, Homo sapiens
NIKGSPWKGSLLLLLVSNLLLCQSVAP

SEQ ID NO: 39 - DNA, 1341 bp, Artificial Sequence
  synthetic
atggattggacctggattctgttcctggtggccgctgccacaagagtgcatagccagggccaagaccggcacatgatccggatgagacagctgatcgacatcgtggaccagctgaagaactacgtgaacgacctggtgcctgagttcctgcctgctcctgaggacgtggaaacaaattgcgagtggtccgccttcagctgcttccagaaggcccagctgaaaagcgccaacaccggcaacaacgagcggatcatcaacgtgtccatcaagaagctgaagcggaagcctcctagcaccaatgccggaagaaggcagaagcacagactgacctgtcctagctgcgacagctacgagaagaagcctccaaaagagttcctggaacggttcaagagcctgctgcagaagatgatccaccagcacctgagcagcagaacccacggctctgaagattctagcggaggcggaggaagtggtggcggaggttctggtggcggtggatcaggcggtggcggatctggcggcggaggcagtggcggaggtggaagcggtggtggtggctctggcggaggcggtagcggcggaggcggatctcttcagatctatatttgggcccctctggccggaacatgtggcgtgttgctgctgtctctggttatcaccggcagcggcgccacaaatttcagcctgctgaaacaggccggcgacgtggaagagaatcctggacctatggactggacttggatactctttctggtcgctgccgccacacgggtgcactctaattgggtcaacgtgatcagcgacctgaagaagatcgaggacctgatccagagcatgcacatcgacgccacactgtacaccgagtccgatgtgcaccctagctgcaaagtgaccgccatgaagtgctttctgctggaactgcaagtgatcagcctggaaagcggcgacgccagcatccacgataccgtggaaaatctgatcatcctggccaacaacagcctgtccagcaacggcaatgtgaccgagagcggctgcaaagagtgcgaggaactggaagagaagaacatcaaagagtttctgcagagcttcgtccacatcgtgcagatgttcatcaacacctcatcaggcggcggtggtagtggaggcggaggctcaggcggcggaggttccggaggtggcggttccggcggaggatctcttcaattgctgcctagctgggccatcacactgatctccgtgaacggcatcttcgtgatctgctgcctgacctactgcttcgcccctagatgcagagagcggagaagaaacgagcggctgagaagagaaagcgtgcggcctgtg

SEQ ID NO: 40 - DNA, 1344 bp, Artificial Sequence
  synthetic
atggattggacctggattctgttcctggtggccgctgccacaagagtgcatagccagggccaagaccggcacatgatccggatgagacagctgatcgacatcgtggaccagctgaagaactacgtgaacgacctggtgcctgagttcctgcctgctcctgaggacgtggaaacaaattgcgagtggtccgccttcagctgcttccagaaggcccagctgaaaagcgccaacaccggcaacaacgagcggatcatcaacgtgtccatcaagaagctgaagcggaagcctcctagcaccaatgccggaagaaggcagaagcacagactgacctgtcctagctgcgacagctacgagaagaagcctccaaaagagttcctggaacggttcaagagcctgctgcagaagatgatccaccagcacctgagcagcagaacccacggctctgaagattctagcggaggcggaggaagtggtggcggaggttctggtggcggtggatcaggcggtggcggatctggcggcggaggcagtggcggaggtggaagcggtggtggtggctctggcggaggcggtagcggcggaggcggatctcttcagatctatatttgggcccctctggccggaacatgtggcgtgttgctgctgtctctggttatcaccggctccggccagtgtaccaattacgccctgcttaaactggccggcgacgtggaatccaatcctggacctatggactggacttggatactctttctggtcgctgccgccacacgggtgcactctaattgggtcaacgtgatcagcgacctgaagaagatcgaggacctgatccagagcatgcacatcgacgccacactgtacaccgagtccgatgtgcaccctagctgcaaagtgaccgccatgaagtgctttctgctggaactgcaagtgatcagcctggaaagcggcgacgccagcatccacgataccgtggaaaatctgatcatcctggccaacaacagcctgtccagcaacggcaatgtgaccgagagcggctgcaaagagtgcgaggaactggaagagaagaacatcaaagagtttctgcagagcttcgtccacatcgtgcagatgttcatcaacacctcatcaggcggcggtggtagtggaggcggaggctcaggcggcggaggttccggaggtggcggttccggcggaggatctcttcaattgctgcctagctgggccatcacactgatctccgtgaacggcatcttcgtgatctgctgcctgacctactgcttcgcccctagatgcagagagcggagaagaaacgagcggctgagaagagaaagcgtgcggcctgtg

SEQ ID NO: 41 - DNA, 1338 bp, Artificial Sequence
  synthetic
atggattggacctggattctgttcctggtggccgctgccacaagagtgcatagccagggccaagaccggcacatgatccggatgagacagctgatcgacatcgtggaccagctgaagaactacgtgaacgacctggtgcctgagttcctgcctgctcctgaggacgtggaaacaaattgcgagtggtccgccttcagctgcttccagaaggcccagctgaaaagcgccaacaccggcaacaacgagcggatcatcaacgtgtccatcaagaagctgaagcggaagcctcctagcaccaatgccggaagaaggcagaagcacagactgacctgtcctagctgcgacagctacgagaagaagcctccaaaagagttcctggaacggttcaagagcctgctgcagaagatgatccaccagcacctgagcagcagaacccacggctctgaagattctagcggaggcggaggaagtggtggcggaggttctggtggcggtggatcaggcggtggcggatctggcggcggaggcagtggcggaggtggaagcggtggtggtggctctggcggaggcggtagcggcggaggcggatctcttcagatctatatttgggcccctctggccggaacatgtggcgtgttgctgctgtctctggttatcaccggttctggcgaaggcagaggctctctgcttacttgtggcgacgtggaagagaatcctggacctatggactggacttggatactctttctggtcgctgccgccacacgggtgcactctaattgggtcaacgtgatcagcgacctgaagaagatcgaggacctgatccagagcatgcacatcgacgccacactgtacaccgagtccgatgtgcaccctagctgcaaagtgaccgccatgaagtgctttctgctggaactgcaagtgatcagcctggaaagcggcgacgccagcatccacgataccgtggaaaatctgatcatcctggccaacaacagcctgtccagcaacggcaatgtgaccgagagcggctgcaaagagtgcgaggaactggaagagaagaacatcaaagagtttctgcagagcttcgtccacatcgtgcagatgttcatcaacacctcatcaggcggcggtggtagtggaggcggaggctcaggcggcggaggttccggaggtggcggttccggcggaggatctcttcaattgctgcctagctgggccatcacactgatctccgtgaacggcatcttcgtgatctgctgcctgacctactgcttcgcccctagatgcagagagcggagaagaaacgagcggctgagaagagaaagcgtgcggcctgtg

SEQ ID NO: 42 - DNA, 1356 bp, Artificial Sequence
  synthetic
atggattggacctggattctgttcctggtggccgctgccacaagagtgcatagccagggccaagaccggcacatgatccggatgagacagctgatcgacatcgtggaccagctgaagaactacgtgaacgacctggtgcctgagttcctgcctgctcctgaggacgtggaaacaaattgcgagtggtccgccttcagctgcttccagaaggcccagctgaaaagcgccaacaccggcaacaacgagcggatcatcaacgtgtccatcaagaagctgaagcggaagcctcctagcaccaatgccggaagaaggcagaagcacagactgacctgtcctagctgcgacagctacgagaagaagcctccaaaagagttcctggaacggttcaagagcctgctgcagaagatgatccaccagcacctgagcagcagaacccacggctctgaagattctagcggaggcggaggaagtggtggcggaggttctggtggcggtggatcaggcggtggcggatctggcggcggaggcagtggcggaggtggaagcggtggtggtggctctggcggaggcggtagcggcggaggcggatctcttcagatctatatttgggcccctctggccggaacatgtggcgtgttgctgctgtctctggttatcaccagggccaaaagaagcggcagcggcgccacaaatttcagcctgctgaaacaggccggcgacgtggaagagaatcctggacctatggactggacttggatactctttctggtcgctgccgccacacgggtgcactctaattgggtcaacgtgatcagcgacctgaagaagatcgaggacctgatccagagcatgcacatcgacgccacactgtacaccgagtccgatgtgcaccctagctgcaaagtgaccgccatgaagtgctttctgctggaactgcaagtgatcagcctggaaagcggcgacgccagcatccacgataccgtggaaaatctgatcatcctggccaacaacagcctgtccagcaacggcaatgtgaccgagagcggctgcaaagagtgcgaggaactggaagagaagaacatcaaagagtttctgcagagcttcgtccacatcgtgcagatgttcatcaacacctcatcaggcggcggtggtagtggaggcggaggctcaggcggcggaggttccggaggtggcggttccggcggaggatctcttcaattgctgcctagctgggccatcacactgatctccgtgaacggcatcttcgtgatctgctgcctgacctactgcttcgcccctagatgcagagagcggagaagaaacgagcggctgagaagagaaagcgtgcggcctgtg

SEQ ID NO: 43 - DNA, 1419 bp, Artificial Sequence
  synthetic
atggattggacctggattctgttcctggtggccgctgccacaagagtgcatagccagggccaagaccggcacatgatccggatgagacagctgatcgacatcgtggaccagctgaagaactacgtgaacgacctggtgcctgagttcctgcctgctcctgaggacgtggaaacaaattgcgagtggtccgccttcagctgcttccagaaggcccagctgaaaagcgccaacaccggcaacaacgagcggatcatcaacgtgtccatcaagaagctgaagcggaagcctcctagcaccaatgccggaagaaggcagaagcacagactgacctgtcctagctgcgacagctacgagaagaagcctccaaaagagttcctggaacggttcaagagcctgctgcagaagatgatccaccagcacctgagcagcagaacccacggctctgaagattctagcggaggcggaggaagtggtggcggaggttctggtggcggtggatcaggcggtggcggatctggcggcggaggcagtggcggaggtggaagcggtggtggtggctctggcggaggcggtagcggcggaggcggatctcttcaattgctgcctagctgggccatcacactgatctccgtgaacggcatcttcgtgatctgctgcctgacctactgcttcgcccctagatgcagagagcggagaagaaacgagcggctgagaagagaatctgtgcggcctgttggctccggccagtgtacaaattatgccctgctgaagctggccggcgacgtggaatctaatcctggacctatggactggacttggatactctttctggtcgctgccgccacacgggtgcactctaattgggtcaacgtgatcagcgacctgaagaagatcgaggacctgatccagagcatgcacatcgacgccacactgtacaccgagtccgatgtgcaccctagctgcaaagtgaccgccatgaagtgctttctgctggaactgcaagtgatcagcctggaaagcggcgacgccagcatccacgataccgtggaaaatctgatcatcctggccaacaacagcctgtccagcaacggcaatgtgaccgagagcggctgcaaagagtgcgaggaactggaagaaaagaacatcaaagagtttctgcagagcttcgtccacatcgtgcagatgttcatcaacacctcatcaggtggcggtggaagcggaggtggcggtagtggcggcggaggctcaggcggcggaggttccggcggaggatctcttcagctcctgccatcttgggctatcaccctgattagtgtgaatgggatctttgtcatctgttgtctcacgtactgtttcgctccccggtgcagagagagaaggcgcaacgaaagactgcggagagaaagcgtcagacccgtg

SEQ ID NO: 44 - DNA, 1431 bp, Artificial Sequence
  synthetic
atggattggacctggattctgttcctggtggccgctgccacaagagtgcatagccagggccaagaccggcacatgatccggatgagacagctgatcgacatcgtggaccagctgaagaactacgtgaacgacctggtgcctgagttcctgcctgctcctgaggacgtggaaacaaattgcgagtggtccgccttcagctgcttccagaaggcccagctgaaaagcgccaacaccggcaacaacgagcggatcatcaacgtgtccatcaagaagctgaagcggaagcctcctagcaccaatgccggaagaaggcagaagcacagactgacctgtcctagctgcgacagctacgagaagaagcctccaaaagagttcctggaacggttcaagagcctgctgcagaagatgatccaccagcacctgagcagcagaacccacggctctgaagattctagcggaggcggaggaagtggtggcggaggttctggtggcggtggatcaggcggtggcggatctggcggcggaggcagtggcggaggtggaagcggtggtggtggctctggcggaggcggtagcggcggaggcggatctcttcaattgctgcctagctgggccatcacactgatctccgtgaacggcatcttcgtgatctgctgcctgacctactgcttcgcccctagatgcagagagcggagaagaaacgagcggctgagaagagaatctgtgcggcctgttagagccaagagatctggaagcggcgccaccaactttagcctgctgaaacaggctggcgacgtggaagagaaccctggacctatggactggacttggatactctttctggtcgctgccgccacacgggtgcactctaattgggtcaacgtgatcagcgacctgaagaagatcgaggacctgatccagagcatgcacatcgacgccacactgtacaccgagtccgatgtgcaccctagctgcaaagtgaccgccatgaagtgctttctgctggaactgcaagtgatcagcctggaaagcggcgacgccagcatccacgataccgtggaaaatctgatcatcctggccaacaacagcctgtccagcaacggcaatgtgaccgagagcggctgcaaagagtgcgaggaactggaagaaaagaacatcaaagagtttctgcagagcttcgtccacatcgtgcagatgttcatcaacacctcatcaggtggcggtggaagcggaggtggcggtagtggcggcggaggctcaggcggcggaggttccggcggaggatctcttcagctcctgccatcttgggctatcaccctgattagtgtgaatgggatctttgtcatctgttgtctcacgtactgtttcgctccccggtgcagagagagaaggcgcaacgaaagactgcggagagaaagcgtcagacccgtg